European Patent Specification EP 4 015 647 B1, published August 30, 2023. Title: Multiplexed Single Molecule RNA Visualization with a Two-Probe Proximity Ligation System. Applicant: The Board of Trustees of The Leland Stanford Junior University. Application EP. The sequence listing filed with the application follows.

SEQUENCE LISTING (8 sequences)

SEQ ID NO: 1 - DNA, 35 bp, Artificial sequence
  synthetic sequence
ctcatcagcacagctatgatgataatgtttatctt

SEQ ID NO: 2 - DNA, 58 bp, Artificial sequence
  synthetic sequence
cattaaaatcctagcacagggactcgcgaattaagtcttagagagagagagaagataa

SEQ ID NO: 3 - DNA, 70 bp, Artificial sequence
  synthetic sequence
atggccataagtggagtccctgtgctaggatttttcatcatagctgtgctgatgagcgctcaggaatcat

SEQ ID NO: 4 - DNA, 168 bp, Artificial sequence
  synthetic sequence
ctcatcagcacagctatgatgataatgttatccgcttcctctctctctctaaagacttaatcgcgcccctgtgctaggataatgtttatcttgcctctctctctctaatcgcgagtccctgtgctaggataatgtttatcttctctctctctctctaaactctctctc

SEQ ID NO: 5 - DNA, 12 bp, Artificial sequence
  synthetic sequence
gcgattaagtct

SEQ ID NO: 6 - DNA, 136 bp, Artificial sequence
  synthetic sequence
tctctgtgctaggataatctttatcttctctctctctctaagacttaatcccctgtgctaggataatctttatcttctctctctctctaagacttaatcgcgagtcccctgtgctaggagataatgtttatcttta

SEQ ID NO: 7 - DNA, 53 bp, Artificial sequence
  synthetic sequence
cattaaatcctagcacagggactcattatcactgaaacatacactaaagataa

SEQ ID NO: 8 - DNA, 10 bp, Artificial sequence
  synthetic sequence
ctataagtct